European Patent Specification EP 4 359 425 B1, published August 5, 2026. Title: Regenerative Polypeptides and Uses Thereof. Applicant: Juvena Therapeutics, Inc. The sequence listing filed with the application follows.

SEQUENCE LISTING (60 sequences)

SEQ ID NO: 1 - DNA, 66 bp, Artificial Sequence
  Signal peptide
atgggagccgcccgcctgctgcccaacctcactctgtgcttacagctgctgattctctgctgtcaa

SEQ ID NO: 2 - DNA, 54 bp, Artificial Sequence
  Signal peptide
atggggctggcctggggactaggcgtcctgttcctgatgcatgtgtgtggcacc

SEQ ID NO: 3 - DNA, 72 bp, Artificial Sequence
  Signal peptide
atgggaatcccaatggggaagtcgatgctggtgcttctcaccttcttggccttcgcctcgtgctgcattgct

SEQ ID NO: 4 - DNA, 87 bp, Artificial Sequence
  Signal peptide
atgcacgtgcgctcactgcgagctgcggcgccgcacagcttcgtggcgctctgggcacccctgttcctgctgcgctccgccctggcc

SEQ ID NO: 5 - DNA, 54 bp, Artificial Sequence
  Signal peptide
atgaagtgggtaacctttatttcccttctttttctctttagctcggcttattcc

SEQ ID NO: 6 - DNA, 57 bp, Artificial Sequence
  Signal peptide
atgacccggctgacagtcctggccctgctggctggtctgctggcgtcctcgagggcc

SEQ ID NO: 7 - DNA, 54 bp, Artificial Sequence
  Signal peptide
atgagggcctggatcttctttctcctttgcctggccgggagggctctggcagca

SEQ ID NO: 8 - DNA, 51 bp, Artificial Sequence
  Signal peptide
atgggagtcaaagttctgtttgccctgatctgcatcgctgtggccgaggcc

SEQ ID NO: 9 - protein, 22 aa, Artificial Sequence
  Signal peptide
MGAARLLPNLTLCLQLLILCCQ

SEQ ID NO: 10 - protein, 18 aa, Artificial Sequence
  Signal peptide
MGLAWGLGVLFLMHVCGT

SEQ ID NO: 11 - protein, 24 aa, Artificial Sequence
  Signal peptide
MGIPMGKSMLVLLTFLAFASCCIA

SEQ ID NO: 12 - protein, 29 aa, Artificial Sequence
  Signal peptide
MHVRSLRAAAPHSFVALWAPLFLLRSALA

SEQ ID NO: 13 - protein, 18 aa, Artificial Sequence
  Signal peptide
MKWVTFISLLFLFSSAYS

SEQ ID NO: 14 - protein, 19 aa, Artificial Sequence
  Signal peptide
MTRLTVLALLAGLLASSRA

SEQ ID NO: 15 - protein, 18 aa, Artificial Sequence
  Signal peptide
MRAWIFFLLCLAGRALAA

SEQ ID NO: 16 - protein, 17 aa, Artificial Sequence
  Signal peptide
MGVKVLFALICIAVAEA

SEQ ID NO: 17 - DNA, 201 bp, Homo sapiens
gcttaccgccccagtgagaccctgtgcggcggggagctggtggacaccctccagttcgtctgtggggaccgcggcttctacttcagcaggcccgcaagccgtgtgagccgtcgcagccgtggcatcgttgaggagtgctgtttccgcagctgtgacctggccctcctggagacgtactgtgctacccccgccaagtccgag

SEQ ID NO: 18 - DNA, 894 bp, Artificial Sequence
  Fusion protein
gcttaccgccccagtgagaccctgtgcggcggggagctggtggacaccctccagttcgtctgtggggaccgcggcttctacttcagcaggcccgcaagccgtgtgagccgtcgcagccgtggcatcgttgaggagtgctgtttccgcagctgtgacctggccctcctggagacgtactgtgctacccccgccaagtccgagggatcgggatcggacaaaactcacacatgcccaccgtgcccagcacctgaagctgccgggggaccgtcagtcttcctcttccccccaaaacccaaggacaccctcatgatctcccggacccctgaggtcacatgcgtggtggtggacgtgagccacgaagaccctgaggtcaagttcaactggtacgtggacggcgtggaggtgcataatgccaagacaaagccgcgggaggagcagtacaacagcacgtaccgtgtggtcagcgtcctcaccgtcctgcaccaggactggctgaatggcaaggagtacaagtgcaaggtctccaacaaagccctcggcgcccccatcgagaaaaccatctccaaagccaaagggcagccccgagaaccacaggtgtacaccctgcccccatcccgggatgagctgaccaagaaccaggtcagcctgacctgcctggtcaaaggcttctatcccagcgacatcgccgtggagtgggagagcaatgggcagccggagaacaactacaagaccacgcctcccgtgctggactccgacggctccttcttcctctacagcaagctcaccgtggacaagagcaggtggcagcaggggaacgtcttctcatgctccgtgatgcatgaggctctgcacaaccactacacgcagaaaagcctctccctgtctccgggtaaa

SEQ ID NO: 19 - DNA, 897 bp, Artificial Sequence
  Fusion protein
gcttaccgccccagtgagaccctgtgcggcggggagctggtggacaccctccagttcgtctgtggggaccgcggcttctacttcagcaggcccgcaagccgtgtgagccgtcgcagccgtggcatcgttgaggagtgctgtttccgcagctgtgacctggccctcctggagacgtactgtgctacccccgccaagtccgagggatctgggagcgctgacaaaactcacacatgcccaccgtgcccagcacctgaagctgccgggggaccgtcagtcttcctcttccccccaaaacccaaggacaccctcatgatctcccggacccctgaggtcacatgcgtggtggtggacgtgagccacgaagaccctgaggtcaagttcaactggtacgtggacggcgtggaggtgcataatgccaagacaaagccgcgggaggagcagtacaacagcacgtaccgtgtggtcagcgtcctcaccgtcctgcaccaggactggctgaatggcaaggagtacaagtgcaaggtctccaacaaagccctcggcgcccccatcgagaaaaccatctccaaagccaaagggcagccccgagaaccacaggtgtacaccctgcccccatcccgggatgagctgaccaagaaccaggtcagcctgacctgcctggtcaaaggcttctatcccagcgacatcgccgtggagtgggagagcaatgggcagccggagaacaactacaagaccacgcctcccgtgctggactccgacggctccttcttcctctacagcaagctcaccgtggacaagagcaggtggcagcaggggaacgtcttctcatgctccgtgatgcatgaggctctgcacaaccactacacgcagaaaagcctctccctgtctccgggtaaa

SEQ ID NO: 20 - DNA, 2025 bp, Artificial Sequence
  Fusion protein
caccatcaccatcaccatagcggcgatgcacacaagagtgaggttgctcatcggtttaaagatttgggagaagaaaatttcaaagccttggtgttgattgcctttgctcagtatcttcagcagtgtccatttgaagatcatgtaaaattagtgaatgaagtaactgaatttgcaaaaacatgtgttgctgatgagtcagctgaaaattgtgacaaatcacttcataccctttttggagacaaattatgcacagttgcaactcttcgtgaaacctatggtgaaatggctgactgctgtgcaaaacaagaacctgagagaaatgaatgcttcttgcaacacaaagatgacaacccaaacctcccccgattggtgagaccagaggttgatgtgatgtgcactgcttttcatgacaatgaagagacatttttgaaaaaatacttatatgaaattgccagaagacatccttacttttatgccccggaactccttttctttgctaaaaggtataaagctgcttttacagaatgttgccaagctgctgataaagctgcctgcctgttgccaaagctcgatgaacttcgggatgaagggaaggcttcgtctgccaaacagagactcaagtgtgccagtctccaaaaatttggagaaagagctttcaaagcatgggcagtagctcgcctgagccagagatttcccaaagctgagtttgcagaagtttccaagttagtgacagatcttaccaaagtccacacggaatgctgccatggagatctgcttgaatgtgctgatgacagggcggaccttgccaagtatatctgtgaaaatcaagattcgatctccagtaaactgaaggaatgctgtgaaaaacctctgttggaaaaatcccactgcattgccgaagtggaaaatgatgagatgcctgctgacttgccttcattagctgctgattttgttgaaagtaaggatgtttgcaaaaactatgctgaggcaaaggatgtcttcctgggcatgtttttgtatgaatatgcaagaaggcatcctgattactctgtcgtgctgctgctgagacttgccaagacatatgaaaccactctagagaagtgctgtgccgctgcagatcctcatgaatgctatgccaaagtgttcgatgaatttaaacctcttgtggaagagcctcagaatttaatcaaacaaaattgtgagctttttgagcagcttggagagtacaaattccagaatgcgctattagttcgttacaccaagaaagtaccccaagtgtcaactccaactcttgtagaggtctcaagaaacctaggaaaagtgggcagcaaatgttgtaaacatcctgaagcaaaaagaatgccctgtgcagaagactatctatccgtggtcctgaaccagttatgtgtgttgcatgagaaaacgccagtaagtgacagagtcaccaaatgctgcacagaatccttggtgaacaggcgaccatgcttttcagctctggaagtcgatgaaacatacgttcccaaagagtttaatgctgaaacattcaccttccatgcagatatatgcacactttctgagaaggagagacaaatcaagaaacaaactgcacttgttgagctcgtgaaacacaagcccaaggcaacaaaagagcaactgaaagctgttatggatgatttcgcagcttttgtagagaagtgctgcaaggctgacgataaggagacctgctttgccgaggagggtaaaaaacttgttgctgcaagtcaagctgccttaggcttaggcggaggcggtagcggaggcggtggctccggtggcggagggtctgcttaccgccccagtgagaccctgtgcggcggggagctggtggacaccctccagttcgtctgtggggaccgcggcttctacttcagcaggcccgcaagccgtgtgagccgtcgcagccgtggcatcgttgaggagtgctgtttccgcagctgtgacctggccctcctggagacgtactgtgctacccccgccaagtccgag

SEQ ID NO: 21 - DNA, 2025 bp, Artificial Sequence
  Fusion protein
caccatcaccatcaccatagcggcgatgcacacaagagtgaggttgctcatcggtttaaagatttgggagaagaaaatttcaaagccttggtgttgattgcctttgctcagtatcttcagcagtgtccatttgaagatcatgtaaaattagtgaatgaagtaactgaatttgcaaaaacatgtgttgctgatgagtcagctgaaaattgtgacaaatcacttcataccctttttggagacaaattatgcacagttgcaactcttcgtgaaacctatggtgaaatggctgactgctgtgcaaaacaagaacctgagagaaatgaatgcttcttgcaacacaaagatgacaacccaaacctcccccgattggtgagaccagaggttgatgtgatgtgcactgcttttcatgacaatgaagagacatttttgaaaaaatacttatatgaaattgccagaagacatccttacttttatgccccggaactccttttctttgctaaaaggtataaagctgcttttacagaatgttgccaagctgctgataaagctgcctgcctgttgccaaagctcgatgaacttcgggatgaagggaaggcttcgtctgccaaacagagactcaagtgtgccagtctccaaaaatttggagaaagagctttcaaagcatgggcagtagctcgcctgagccagagatttcccaaagctgagtttgcagaagtttccaagttagtgacagatcttaccaaagtccacacggaatgctgccatggagatctgcttgaatgtgctgatgacagggcggaccttgccaagtatatctgtgaaaatcaagattcgatctccagtaaactgaaggaatgctgtgaaaaacctctgttggaaaaatcccactgcattgccgaagtggaaaatgatgagatgcctgctgacttgccttcattagctgctgattttgttgaaagtaaggatgtttgcaaaaactatgctgaggcaaaggatgtcttcctgggcatgtttttgtatgaatatgcaagaaggcatcctgattactctgtcgtgctgctgctgagacttgccaagacatatgaaaccactctagagaagtgctgtgccgctgcagatcctcatgaatgctatgccaaagtgttcgatgaatttaaacctcttgtggaagagcctcagaatttaatcaaacaaaattgtgagctttttgagcagcttggagagtacaaattccagaatgcgctattagttcgttacaccaagaaagtaccccaagtgtcaactccaactcttgtagaggtctcaagaaacctaggaaaagtgggcagcaaatgttgtaaacatcctgaagcaaaaagaatgccctgtgcagaagactatctatccgtggtcctgaaccagttatgtgtgttgcatgagaaaacgccagtaagtgacagagtcaccaaatgctgcacagaatccttggtgaacaggcgaccatgcttttcagctctggaagtcgatgaaacatacgttcccaaagagtttaatgctgaaacattcaccttccatgcagatatatgcacactttctgagaaggagagacaaatcaagaaacaaactgcacttgttgagctcgtgaaacacaagcccaaggcaacaaaagagcaactgaaagctgttatggatgatttcgcagcttttgtagagaagtgctgcaaggctgacgataaggagacctgctttgccgaggagggtaaaaaacttgttgctgcaagtcaagctgccttaggcttaggcggaggcggtagcggaggcggtggctccggtggcggagggtctgcttaccgccccagtgagaccctgtgcggcggggagctggtggacaccctccagttcgtctgtggggaccgcggcttctacttcagcaggcccgcaagccgtgtgagcgctcgcagccgtggcatcgttgaggagtgctgtttccgcagctgtgacctggccctcctggagacgtactgtgctacccccgccaagtccgag

SEQ ID NO: 22 - DNA, 2025 bp, Artificial Sequence
  Fusion protein
caccatcaccatcaccatagcggcgatgcacacaagagtgaggttgctcatcggtttaaagatttgggagaagaaaatttcaaagccttggtgttgattgcctttgctcagtatcttcagcagtgtccatttgaagatcatgtaaaattagtgaatgaagtaactgaatttgcaaaaacatgtgttgctgatgagtcagctgaaaattgtgacaaatcacttcataccctttttggagacaaattatgcacagttgcaactcttcgtgaaacctatggtgaaatggctgactgctgtgcaaaacaagaacctgagagaaatgaatgcttcttgcaacacaaagatgacaacccaaacctcccccgattggtgagaccagaggttgatgtgatgtgcactgcttttcatgacaatgaagagacatttttgaaaaaatacttatatgaaattgccagaagacatccttacttttatgccccggaactccttttctttgctaaaaggtataaagctgcttttacagaatgttgccaagctgctgataaagctgcctgcctgttgccaaagctcgatgaacttcgggatgaagggaaggcttcgtctgccaaacagagactcaagtgtgccagtctccaaaaatttggagaaagagctttcaaagcatgggcagtagctcgcctgagccagagatttcccaaagctgagtttgcagaagtttccaagttagtgacagatcttaccaaagtccacacggaatgctgccatggagatctgcttgaatgtgctgatgacagggcggaccttgccaagtatatctgtgaaaatcaagattcgatctccagtaaactgaaggaatgctgtgaaaaacctctgttggaaaaatcccactgcattgccgaagtggaaaatgatgagatgcctgctgacttgccttcattagctgctgattttgttgaaagtaaggatgtttgcaaaaactatgctgaggcaaaggatgtcttcctgggcatgtttttgtatgaatatgcaagaaggcatcctgattactctgtcgtgctgctgctgagacttgccaagacatatgaaaccactctagagaagtgctgtgccgctgcagatcctcatgaatgctatgccaaagtgttcgatgaatttaaacctcttgtggaagagcctcagaatttaatcaaacaaaattgtgagctttttgagcagcttggagagtacaaattccagaatgcgctattagttcgttacaccaagaaagtaccccaagtgtcaactccaactcttgtagaggtctcaagaaacctaggaaaagtgggcagcaaatgttgtaaacatcctgaagcaaaaagaatgccctgtgcagaagactatctatccgtggtcctgaaccagttatgtgtgttgcatgagaaaacgccagtaagtgacagagtcaccaaatgctgcacagaatccttggtgaacaggcgaccatgcttttcagctctggaagtcgatgaaacatacgttcccaaagagtttaatgctgaaacattcaccttccatgcagatatatgcacactttctgagaaggagagacaaatcaagaaacaaactgcacttgttgagctcgtgaaacacaagcccaaggcaacaaaagagcaactgaaagctgttatggatgatttcgcagcttttgtagagaagtgctgcaaggctgacgataaggagacctgctttgccgaggagggtaaaaaacttgttgctgcaagtcaagctgccttaggcttaggcggaggcggtagcggaggcggtggctccggtggcggagggtctgcttaccgccccagtgagaccctgtgcggcggggagctggtggacaccctccagttcgtctgtggggaccgcggcttctacttcagcaggcccgcaagccgtgtgagccagcgcagccgtggcatcgttgaggagtgctgtttccgcagctgtgacctggccctcctggagacgtactgtgctacccccgccaagtccgag

SEQ ID NO: 23 - DNA, 2025 bp, Artificial Sequence
  Fusion protein
caccatcaccatcaccatagcggcgatgcacacaagagtgaggttgctcatcggtttaaagatttgggagaagaaaatttcaaagccttggtgttgattgcctttgctcagtatcttcagcagtgtccatttgaagatcatgtaaaattagtgaatgaagtaactgaatttgcaaaaacatgtgttgctgatgagtcagctgaaaattgtgacaaatcacttcataccctttttggagacaaattatgcacagttgcaactcttcgtgaaacctatggtgaaatggctgactgctgtgcaaaacaagaacctgagagaaatgaatgcttcttgcaacacaaagatgacaacccaaacctcccccgattggtgagaccagaggttgatgtgatgtgcactgcttttcatgacaatgaagagacatttttgaaaaaatacttatatgaaattgccagaagacatccttacttttatgccccggaactccttttctttgctaaaaggtataaagctgcttttacagaatgttgccaagctgctgataaagctgcctgcctgttgccaaagctcgatgaacttcgggatgaagggaaggcttcgtctgccaaacagagactcaagtgtgccagtctccaaaaatttggagaaagagctttcaaagcatgggcagtagctcgcctgagccagagatttcccaaagctgagtttgcagaagtttccaagttagtgacagatcttaccaaagtccacacggaatgctgccatggagatctgcttgaatgtgctgatgacagggcggaccttgccaagtatatctgtgaaaatcaagattcgatctccagtaaactgaaggaatgctgtgaaaaacctctgttggaaaaatcccactgcattgccgaagtggaaaatgatgagatgcctgctgacttgccttcattagctgctgattttgttgaaagtaaggatgtttgcaaaaactatgctgaggcaaaggatgtcttcctgggcatgtttttgtatgaatatgcaagaaggcatcctgattactctgtcgtgctgctgctgagacttgccaagacatatgaaaccactctagagaagtgctgtgccgctgcagatcctcatgaatgctatgccaaagtgttcgatgaatttaaacctcttgtggaagagcctcagaatttaatcaaacaaaattgtgagctttttgagcagcttggagagtacaaattccagaatgcgctattagttcgttacaccaagaaagtaccccaagtgtcaactccaactcttgtagaggtctcaagaaacctaggaaaagtgggcagcaaatgttgtaaacatcctgaagcaaaaagaatgccctgtgcagaagactatctatccgtggtcctgaaccagttatgtgtgttgcatgagaaaacgccagtaagtgacagagtcaccaaatgctgcacagaatccttggtgaacaggcgaccatgcttttcagctctggaagtcgatgaaacatacgttcccaaagagtttaatgctgaaacattcaccttccatgcagatatatgcacactttctgagaaggagagacaaatcaagaaacaaactgcacttgttgagctcgtgaaacacaagcccaaggcaacaaaagagcaactgaaagctgttatggatgatttcgcagcttttgtagagaagtgctgcaaggctgacgataaggagacctgctttgccgaggagggtaaaaaacttgttgctgcaagtcaagctgccttaggcttaggcggaggcggtagcggaggcggtggctccggtggcggagggtctgcttaccgccccagtgagaccctgtgcggcggggagctggtggacaccctccagttcgtctgtggggaccgcggcttctacttcagcaggcccgcaagccgtgtgagccgtcgcagcgctggcatcgttgaggagtgctgtttccgcagctgtgacctggccctcctggagacgtactgtgctacccccgccaagtccgag

SEQ ID NO: 24 - DNA, 2025 bp, Artificial Sequence
  Fusion protein
caccatcaccatcaccatagcggcgatgcacacaagagtgaggttgctcatcggtttaaagatttgggagaagaaaatttcaaagccttggtgttgattgcctttgctcagtatcttcagcagtgtccatttgaagatcatgtaaaattagtgaatgaagtaactgaatttgcaaaaacatgtgttgctgatgagtcagctgaaaattgtgacaaatcacttcataccctttttggagacaaattatgcacagttgcaactcttcgtgaaacctatggtgaaatggctgactgctgtgcaaaacaagaacctgagagaaatgaatgcttcttgcaacacaaagatgacaacccaaacctcccccgattggtgagaccagaggttgatgtgatgtgcactgcttttcatgacaatgaagagacatttttgaaaaaatacttatatgaaattgccagaagacatccttacttttatgccccggaactccttttctttgctaaaaggtataaagctgcttttacagaatgttgccaagctgctgataaagctgcctgcctgttgccaaagctcgatgaacttcgggatgaagggaaggcttcgtctgccaaacagagactcaagtgtgccagtctccaaaaatttggagaaagagctttcaaagcatgggcagtagctcgcctgagccagagatttcccaaagctgagtttgcagaagtttccaagttagtgacagatcttaccaaagtccacacggaatgctgccatggagatctgcttgaatgtgctgatgacagggcggaccttgccaagtatatctgtgaaaatcaagattcgatctccagtaaactgaaggaatgctgtgaaaaacctctgttggaaaaatcccactgcattgccgaagtggaaaatgatgagatgcctgctgacttgccttcattagctgctgattttgttgaaagtaaggatgtttgcaaaaactatgctgaggcaaaggatgtcttcctgggcatgtttttgtatgaatatgcaagaaggcatcctgattactctgtcgtgctgctgctgagacttgccaagacatatgaaaccactctagagaagtgctgtgccgctgcagatcctcatgaatgctatgccaaagtgttcgatgaatttaaacctcttgtggaagagcctcagaatttaatcaaacaaaattgtgagctttttgagcagcttggagagtacaaattccagaatgcgctattagttcgttacaccaagaaagtaccccaagtgtcaactccaactcttgtagaggtctcaagaaacctaggaaaagtgggcagcaaatgttgtaaacatcctgaagcaaaaagaatgccctgtgcagaagactatctatccgtggtcctgaaccagttatgtgtgttgcatgagaaaacgccagtaagtgacagagtcaccaaatgctgcacagaatccttggtgaacaggcgaccatgcttttcagctctggaagtcgatgaaacatacgttcccaaagagtttaatgctgaaacattcaccttccatgcagatatatgcacactttctgagaaggagagacaaatcaagaaacaaactgcacttgttgagctcgtgaaacacaagcccaaggcaacaaaagagcaactgaaagctgttatggatgatttcgcagcttttgtagagaagtgctgcaaggctgacgataaggagacctgctttgccgaggagggtaaaaaacttgttgctgcaagtcaagctgccttaggcttaggcggaggcggtagcggaggcggtggctccggtggcggagggtctgcttaccgccccagtgagaccctgtgcggcggggagctggtggacaccctccagttcgtctgtggggaccgcggcttctacttcagcaggcccgcaagccgtgtgagccgtcgcagccagggcatcgttgaggagtgctgtttccgcagctgtgacctggccctcctggagacgtactgtgctacccccgccaagtccgag

SEQ ID NO: 25 - DNA, 933 bp, Artificial Sequence
  Fusion protein
gcttaccgccccagtgagaccctgtgcggcggggagctggtggacaccctccagttcgtctgtggggaccgcggcttctacttcagcaggcccgcaagccgtgtgagccgtcgcagccgtggcatcgttgaggagtgctgtttccgcagctgtgacctggccctcctggagacgtactgtgctacccccgccaagtccgagggcggaggcggtagcggaggcggtggctccggtggcggagggtctgagtccaaatatggtcccccatgcccaccctgcccagcacctgagttcctggggggaccatcagtcttcctgttccccccaaaacccaaggacactctcatgatctcccggacccctgaggtcacgtgcgtggtggtggacgtgagccaggaagaccccgaggtccagttcaactggtacgtggatggcgtggaggtgcataatgccaagacaaagccgcgggaggagcagttcaacagcacgtaccgtgtggtcagcgtcctcaccgtcctgcaccaggactggctgaacggcaaggagtacaagtgcaaggtctccaacaaaggcctcccgtcctccatcgagaaaaccatctccaaagccaaagggcagccccgagagccacaggtgtacaccctgcccccatcccaggaggagatgaccaagaaccaggtcagcctgacctgcctggtcaaaggcttctaccccagcgacatcgccgtggagtgggagagcaatgggcagccggagaacaactacaagaccacgcctcccgtgctggactccgacggctccttcttcctctacagcaggctcaccgtggacaagagcaggtggcaggaggggaatgtcttctcatgctccgtgatgcatgaggctctgcacaaccactacacacagaagagcctctccctgtctctgggtaaa

SEQ ID NO: 26 - DNA, 888 bp, Artificial Sequence
  Fusion protein
gcttaccgccccagtgagaccctgtgcggcggggagctggtggacaccctccagttcgtctgtggggaccgcggcttctacttcagcaggcccgcaagccgtgtgagccgtcgcagccgtggcatcgttgaggagtgctgtttccgcagctgtgacctggccctcctggagacgtactgtgctacccccgccaagtccgaggagtccaaatatggtcccccatgcccaccctgcccagcacctgagttcctggggggaccatcagtcttcctgttccccccaaaacccaaggacactctcatgatctcccggacccctgaggtcacgtgcgtggtggtggacgtgagccaggaagaccccgaggtccagttcaactggtacgtggatggcgtggaggtgcataatgccaagacaaagccgcgggaggagcagttcaacagcacgtaccgtgtggtcagcgtcctcaccgtcctgcaccaggactggctgaacggcaaggagtacaagtgcaaggtctccaacaaaggcctcccgtcctccatcgagaaaaccatctccaaagccaaagggcagccccgagagccacaggtgtacaccctgcccccatcccaggaggagatgaccaagaaccaggtcagcctgacctgcctggtcaaaggcttctaccccagcgacatcgccgtggagtgggagagcaatgggcagccggagaacaactacaagaccacgcctcccgtgctggactccgacggctccttcttcctctacagcaggctcaccgtggacaagagcaggtggcaggaggggaatgtcttctcatgctccgtgatgcatgaggctctgcacaaccactacacacagaagagcctctccctgtctctgggtaaa

SEQ ID NO: 27 - DNA, 933 bp, Artificial Sequence
  Fusion protein
gagtccaaatatggtcccccatgcccaccctgcccagcacctgagttcctggggggaccatcagtcttcctgttccccccaaaacccaaggacactctcatgatctcccggacccctgaggtcacgtgcgtggtggtggacgtgagccaggaagaccccgaggtccagttcaactggtacgtggatggcgtggaggtgcataatgccaagacaaagccgcgggaggagcagttcaacagcacgtaccgtgtggtcagcgtcctcaccgtcctgcaccaggactggctgaacggcaaggagtacaagtgcaaggtctccaacaaaggcctcccgtcctccatcgagaaaaccatctccaaagccaaagggcagccccgagagccacaggtgtacaccctgcccccatcccaggaggagatgaccaagaaccaggtcagcctgacctgcctggtcaaaggcttctaccccagcgacatcgccgtggagtgggagagcaatgggcagccggagaacaactacaagaccacgcctcccgtgctggactccgacggctccttcttcctctacagcaggctcaccgtggacaagagcaggtggcaggaggggaatgtcttctcatgctccgtgatgcatgaggctctgcacaaccactacacacagaagagcctctccctgtctctgggtaaaggcggaggcggtagcggaggcggtggctccggtggcggagggtctgcttaccgccccagtgagaccctgtgcggcggggagctggtggacaccctccagttcgtctgtggggaccgcggcttctacttcagcaggcccgcaagccgtgtgagccgtcgcagccgtggcatcgttgaggagtgctgtttccgcagctgtgacctggccctcctggagacgtactgtgctacccccgccaagtccgag

SEQ ID NO: 28 - DNA, 933 bp, Artificial Sequence
  Fusion protein
gcttaccgccccagtgagaccctgtgcggcggggagctggtggacaccctccagttcgtctgtggggaccgcggcttctacttcagcaggcccgcaagccgtgtgagcgctcgcagccgtggcatcgttgaggagtgctgtttccgcagctgtgacctggccctcctggagacgtactgtgctacccccgccaagtccgagggcggaggcggtagcggaggcggtggctccggtggcggagggtctgagtccaaatatggtcccccatgcccaccctgcccagcacctgagttcctggggggaccatcagtcttcctgttccccccaaaacccaaggacactctcatgatctcccggacccctgaggtcacgtgcgtggtggtggacgtgagccaggaagaccccgaggtccagttcaactggtacgtggatggcgtggaggtgcataatgccaagacaaagccgcgggaggagcagttcaacagcacgtaccgtgtggtcagcgtcctcaccgtcctgcaccaggactggctgaacggcaaggagtacaagtgcaaggtctccaacaaaggcctcccgtcctccatcgagaaaaccatctccaaagccaaagggcagccccgagagccacaggtgtacaccctgcccccatcccaggaggagatgaccaagaaccaggtcagcctgacctgcctggtcaaaggcttctaccccagcgacatcgccgtggagtgggagagcaatgggcagccggagaacaactacaagaccacgcctcccgtgctggactccgacggctccttcttcctctacagcaggctcaccgtggacaagagcaggtggcaggaggggaatgtcttctcatgctccgtgatgcatgaggctctgcacaaccactacacacagaagagcctctccctgtctctgggtaaa

SEQ ID NO: 29 - protein, 67 aa, Homo sapiens
AYRPSETLCGGELVDTLQFVCGDRGFYFSRPASRVSRRSRGIVEECCFRSCDLALLETYCATPAKSE

SEQ ID NO: 30 - protein, 298 aa, Artificial Sequence
  Fusion protein
AYRPSETLCGGELVDTLQFVCGDRGFYFSRPASRVSRRSRGIVEECCFRSCDLALLETYCATPAKSEGSGSDKTHTCPPCPAPEAAGGPSVFLFPPKPKDTLMISRTPEVTCVVVDVSHEDPEVKFNWYVDGVEVHNAKTKPREEQYNSTYRVVSVLTVLHQDWLNGKEYKCKVSNKALGAPIEKTISKAKGQPREPQVYTLPPSRDELTKNQVSLTCLVKGFYPSDIAVEWESNGQPENNYKTTPPVLDSDGSFFLYSKLTVDKSRWQQGNVFSCSVMHEALHNHYTQKSLSLSPGK

SEQ ID NO: 31 - protein, 299 aa, Artificial Sequence
  Fusion protein
AYRPSETLCGGELVDTLQFVCGDRGFYFSRPASRVSRRSRGIVEECCFRSCDLALLETYCATPAKSEGSGSADKTHTCPPCPAPEAAGGPSVFLFPPKPKDTLMISRTPEVTCVVVDVSHEDPEVKFNWYVDGVEVHNAKTKPREEQYNSTYRVVSVLTVLHQDWLNGKEYKCKVSNKALGAPIEKTISKAKGQPREPQVYTLPPSRDELTKNQVSLTCLVKGFYPSDIAVEWESNGQPENNYKTTPPVLDSDGSFFLYSKLTVDKSRWQQGNVFSCSVMHEALHNHYTQKSLSLSPGK

SEQ ID NO: 32 - protein, 180 aa, Artificial Sequence
  Fusion protein
MGIPMGKSMLVLLTFLAFASCCIAAYRPSETLCGGELVDTLQFVCGDRGFYFSRPASRVSRRSRGIVEECCFRSCDLALLETYCATPAKSERDVSTPPTVLPDNFPRYPVGKFFQYDTWKQSTQRLRRGLPALLRARRGHVLAKELEAFREAKRHRPLIALPTQDPAHGGAPPEMASNRK

SEQ ID NO: 33 - protein, 675 aa, Artificial Sequence
  Fusion protein
HHHHHHSGDAHKSEVAHRFKDLGEENFKALVLIAFAQYLQQCPFEDHVKLVNEVTEFAKTCVADESAENCDKSLHTLFGDKLCTVATLRETYGEMADCCAKQEPERNECFLQHKDDNPNLPRLVRPEVDVMCTAFHDNEETFLKKYLYEIARRHPYFYAPELLFFAKRYKAAFTECCQAADKAACLLPKLDELRDEGKASSAKQRLKCASLQKFGERAFKAWAVARLSQRFPKAEFAEVSKLVTDLTKVHTECCHGDLLECADDRADLAKYICENQDSISSKLKECCEKPLLEKSHCIAEVENDEMPADLPSLAADFVESKDVCKNYAEAKDVFLGMFLYEYARRHPDYSVVLLLRLAKTYETTLEKCCAAADPHECYAKVFDEFKPLVEEPQNLIKQNCELFEQLGEYKFQNALLVRYTKKVPQVSTPTLVEVSRNLGKVGSKCCKHPEAKRMPCAEDYLSVVLNQLCVLHEKTPVSDRVTKCCTESLVNRRPCFSALEVDETYVPKEFNAETFTFHADICTLSEKERQIKKQTALVELVKHKPKATKEQLKAVMDDFAAFVEKCCKADDKETCFAEEGKKLVAASQAALGLGGGGSGGGGSGGGGSAYRPSETLCGGELVDTLQFVCGDRGFYFSRPASRVSRRSRGIVEECCFRSCDLALLETYCATPAKSE

SEQ ID NO: 34 - protein, 675 aa, Artificial Sequence
  Fusion protein
HHHHHHSGDAHKSEVAHRFKDLGEENFKALVLIAFAQYLQQCPFEDHVKLVNEVTEFAKTCVADESAENCDKSLHTLFGDKLCTVATLRETYGEMADCCAKQEPERNECFLQHKDDNPNLPRLVRPEVDVMCTAFHDNEETFLKKYLYEIARRHPYFYAPELLFFAKRYKAAFTECCQAADKAACLLPKLDELRDEGKASSAKQRLKCASLQKFGERAFKAWAVARLSQRFPKAEFAEVSKLVTDLTKVHTECCHGDLLECADDRADLAKYICENQDSISSKLKECCEKPLLEKSHCIAEVENDEMPADLPSLAADFVESKDVCKNYAEAKDVFLGMFLYEYARRHPDYSVVLLLRLAKTYETTLEKCCAAADPHECYAKVFDEFKPLVEEPQNLIKQNCELFEQLGEYKFQNALLVRYTKKVPQVSTPTLVEVSRNLGKVGSKCCKHPEAKRMPCAEDYLSVVLNQLCVLHEKTPVSDRVTKCCTESLVNRRPCFSALEVDETYVPKEFNAETFTFHADICTLSEKERQIKKQTALVELVKHKPKATKEQLKAVMDDFAAFVEKCCKADDKETCFAEEGKKLVAASQAALGLGGGGSGGGGSGGGGSAYRPSETLCGGELVDTLQFVCGDRGFYFSRPASRVSARSRGIVEECCFRSCDLALLETYCATPAKSE

SEQ ID NO: 35 - protein, 675 aa, Artificial Sequence
  Fusion protein
HHHHHHSGDAHKSEVAHRFKDLGEENFKALVLIAFAQYLQQCPFEDHVKLVNEVTEFAKTCVADESAENCDKSLHTLFGDKLCTVATLRETYGEMADCCAKQEPERNECFLQHKDDNPNLPRLVRPEVDVMCTAFHDNEETFLKKYLYEIARRHPYFYAPELLFFAKRYKAAFTECCQAADKAACLLPKLDELRDEGKASSAKQRLKCASLQKFGERAFKAWAVARLSQRFPKAEFAEVSKLVTDLTKVHTECCHGDLLECADDRADLAKYICENQDSISSKLKECCEKPLLEKSHCIAEVENDEMPADLPSLAADFVESKDVCKNYAEAKDVFLGMFLYEYARRHPDYSVVLLLRLAKTYETTLEKCCAAADPHECYAKVFDEFKPLVEEPQNLIKQNCELFEQLGEYKFQNALLVRYTKKVPQVSTPTLVEVSRNLGKVGSKCCKHPEAKRMPCAEDYLSVVLNQLCVLHEKTPVSDRVTKCCTESLVNRRPCFSALEVDETYVPKEFNAETFTFHADICTLSEKERQIKKQTALVELVKHKPKATKEQLKAVMDDFAAFVEKCCKADDKETCFAEEGKKLVAASQAALGLGGGGSGGGGSGGGGSAYRPSETLCGGELVDTLQFVCGDRGFYFSRPASRVSQRSRGIVEECCFRSCDLALLETYCATPAKSE

SEQ ID NO: 36 - protein, 675 aa, Artificial Sequence
  Fusion protein
HHHHHHSGDAHKSEVAHRFKDLGEENFKALVLIAFAQYLQQCPFEDHVKLVNEVTEFAKTCVADESAENCDKSLHTLFGDKLCTVATLRETYGEMADCCAKQEPERNECFLQHKDDNPNLPRLVRPEVDVMCTAFHDNEETFLKKYLYEIARRHPYFYAPELLFFAKRYKAAFTECCQAADKAACLLPKLDELRDEGKASSAKQRLKCASLQKFGERAFKAWAVARLSQRFPKAEFAEVSKLVTDLTKVHTECCHGDLLECADDRADLAKYICENQDSISSKLKECCEKPLLEKSHCIAEVENDEMPADLPSLAADFVESKDVCKNYAEAKDVFLGMFLYEYARRHPDYSVVLLLRLAKTYETTLEKCCAAADPHECYAKVFDEFKPLVEEPQNLIKQNCELFEQLGEYKFQNALLVRYTKKVPQVSTPTLVEVSRNLGKVGSKCCKHPEAKRMPCAEDYLSVVLNQLCVLHEKTPVSDRVTKCCTESLVNRRPCFSALEVDETYVPKEFNAETFTFHADICTLSEKERQIKKQTALVELVKHKPKATKEQLKAVMDDFAAFVEKCCKADDKETCFAEEGKKLVAASQAALGLGGGGSGGGGSGGGGSAYRPSETLCGGELVDTLQFVCGDRGFYFSRPASRVSRRSAGIVEECCFRSCDLALLETYCATPAKSE

SEQ ID NO: 37 - protein, 675 aa, Artificial Sequence
  Fusion protein
HHHHHHSGDAHKSEVAHRFKDLGEENFKALVLIAFAQYLQQCPFEDHVKLVNEVTEFAKTCVADESAENCDKSLHTLFGDKLCTVATLRETYGEMADCCAKQEPERNECFLQHKDDNPNLPRLVRPEVDVMCTAFHDNEETFLKKYLYEIARRHPYFYAPELLFFAKRYKAAFTECCQAADKAACLLPKLDELRDEGKASSAKQRLKCASLQKFGERAFKAWAVARLSQRFPKAEFAEVSKLVTDLTKVHTECCHGDLLECADDRADLAKYICENQDSISSKLKECCEKPLLEKSHCIAEVENDEMPADLPSLAADFVESKDVCKNYAEAKDVFLGMFLYEYARRHPDYSVVLLLRLAKTYETTLEKCCAAADPHECYAKVFDEFKPLVEEPQNLIKQNCELFEQLGEYKFQNALLVRYTKKVPQVSTPTLVEVSRNLGKVGSKCCKHPEAKRMPCAEDYLSVVLNQLCVLHEKTPVSDRVTKCCTESLVNRRPCFSALEVDETYVPKEFNAETFTFHADICTLSEKERQIKKQTALVELVKHKPKATKEQLKAVMDDFAAFVEKCCKADDKETCFAEEGKKLVAASQAALGLGGGGSGGGGSGGGGSAYRPSETLCGGELVDTLQFVCGDRGFYFSRPASRVSRRSQGIVEECCFRSCDLALLETYCATPAKSE

SEQ ID NO: 38 - protein, 311 aa, Artificial Sequence
  Fusion protein
AYRPSETLCGGELVDTLQFVCGDRGFYFSRPASRVSRRSRGIVEECCFRSCDLALLETYCATPAKSEGGGGSGGGGSGGGGSESKYGPPCPPCPAPEFLGGPSVFLFPPKPKDTLMISRTPEVTCVVVDVSQEDPEVQFNWYVDGVEVHNAKTKPREEQFNSTYRVVSVLTVLHQDWLNGKEYKCKVSNKGLPSSIEKTISKAKGQPREPQVYTLPPSQEEMTKNQVSLTCLVKGFYPSDIAVEWESNGQPENNYKTTPPVLDSDGSFFLYSRLTVDKSRWQEGNVFSCSVMHEALHNHYTQKSLSLSLGK

SEQ ID NO: 39 - protein, 296 aa, Artificial Sequence
  Fusion protein
AYRPSETLCGGELVDTLQFVCGDRGFYFSRPASRVSRRSRGIVEECCFRSCDLALLETYCATPAKSEESKYGPPCPPCPAPEFLGGPSVFLFPPKPKDTLMISRTPEVTCVVVDVSQEDPEVQFNWYVDGVEVHNAKTKPREEQFNSTYRVVSVLTVLHQDWLNGKEYKCKVSNKGLPSSIEKTISKAKGQPREPQVYTLPPSQEEMTKNQVSLTCLVKGFYPSDIAVEWESNGQPENNYKTTPPVLDSDGSFFLYSRLTVDKSRWQEGNVFSCSVMHEALHNHYTQKSLSLSLGK

SEQ ID NO: 40 - protein, 311 aa, Artificial Sequence
  Fusion protein
ESKYGPPCPPCPAPEFLGGPSVFLFPPKPKDTLMISRTPEVTCVVVDVSQEDPEVQFNWYVDGVEVHNAKTKPREEQFNSTYRVVSVLTVLHQDWLNGKEYKCKVSNKGLPSSIEKTISKAKGQPREPQVYTLPPSQEEMTKNQVSLTCLVKGFYPSDIAVEWESNGQPENNYKTTPPVLDSDGSFFLYSRLTVDKSRWQEGNVFSCSVMHEALHNHYTQKSLSLSLGKGGGGSGGGGSGGGGSAYRPSETLCGGELVDTLQFVCGDRGFYFSRPASRVSRRSRGIVEECCFRSCDLALLETYCATPAKSE

SEQ ID NO: 41 - protein, 311 aa, Artificial Sequence
  Fusion protein
AYRPSETLCGGELVDTLQFVCGDRGFYFSRPASRVSARSRGIVEECCFRSCDLALLETYCATPAKSEGGGGSGGGGSGGGGSESKYGPPCPPCPAPEFLGGPSVFLFPPKPKDTLMISRTPEVTCVVVDVSQEDPEVQFNWYVDGVEVHNAKTKPREEQFNSTYRVVSVLTVLHQDWLNGKEYKCKVSNKGLPSSIEKTISKAKGQPREPQVYTLPPSQEEMTKNQVSLTCLVKGFYPSDIAVEWESNGQPENNYKTTPPVLDSDGSFFLYSRLTVDKSRWQEGNVFSCSVMHEALHNHYTQKSLSLSLGK

SEQ ID NO: 42 - protein, 17 aa, Artificial Sequence
  Portion of IGF2
RGFYFSRPASRVSRRSR

SEQ ID NO: 43 - DNA, 12 bp, Artificial Sequence
  Short flexible linker
ggatcgggatcg

SEQ ID NO: 44 - DNA, 15 bp, Artificial Sequence
  Short flexible linker
ggatctgggagcgct

SEQ ID NO: 45 - DNA, 45 bp, Artificial Sequence
  Long flexible linker
ggcggaggcggtagcggaggcggtggctccggtggcggagggtct

SEQ ID NO: 46 - DNA, 681 bp, Artificial Sequence
  Fusion protein
gacaaaactcacacatgcccaccgtgcccagcacctgaagctgccgggggaccgtcagtcttcctcttccccccaaaacccaaggacaccctcatgatctcccggacccctgaggtcacatgcgtggtggtggacgtgagccacgaagaccctgaggtcaagttcaactggtacgtggacggcgtggaggtgcataatgccaagacaaagccgcgggaggagcagtacaacagcacgtaccgtgtggtcagcgtcctcaccgtcctgcaccaggactggctgaatggcaaggagtacaagtgcaaggtctccaacaaagccctcggcgcccccatcgagaaaaccatctccaaagccaaagggcagccccgagaaccacaggtgtacaccctgcccccatcccgggatgagctgaccaagaaccaggtcagcctgacctgcctggtcaaaggcttctatcccagcgacatcgccgtggagtgggagagcaatgggcagccggagaacaactacaagaccacgcctcccgtgctggactccgacggctccttcttcctctacagcaagctcaccgtggacaagagcaggtggcagcaggggaacgtcttctcatgctccgtgatgcatgaggctctgcacaaccactacacgcagaaaagcctctccctgtctccgggtaaa

SEQ ID NO: 47 - DNA, 687 bp, Artificial Sequence
  Fusion protein
gagtccaaatatggtcccccatgcccaccctgcccagcacctgagttcctggggggaccatcagtcttcctgttccccccaaaacccaaggacactctcatgatctcccggacccctgaggtcacgtgcgtggtggtggacgtgagccaggaagaccccgaggtccagttcaactggtacgtggatggcgtggaggtgcataatgccaagacaaagccgcgggaggagcagttcaacagcacgtaccgtgtggtcagcgtcctcaccgtcctgcaccaggactggctgaacggcaaggagtacaagtgcaaggtctccaacaaaggcctcccgtcctccatcgagaaaaccatctccaaagccaaagggcagccccgagagccacaggtgtacaccctgcccccatcccaggaggagatgaccaagaaccaggtcagcctgacctgcctggtcaaaggcttctaccccagcgacatcgccgtggagtgggagagcaatgggcagccggagaacaactacaagaccacgcctcccgtgctggactccgacggctccttcttcctctacagcaggctcaccgtggacaagagcaggtggcaggaggggaatgtcttctcatgctccgtgatgcatgaggctctgcacaaccactacacacagaagagcctctccctgtctctgggtaaa

SEQ ID NO: 48 - DNA, 18 bp, Artificial Sequence
  Six His peptide
caccatcaccatcaccat

SEQ ID NO: 49 - DNA, 24 bp, Artificial Sequence
  Strep-Tactin binding peptide
tggagccacccgcagttcgaaaaa

SEQ ID NO: 50 - DNA, 1755 bp, Homo sapiens
gatgcacacaagagtgaggttgctcatcggtttaaagatttgggagaagaaaatttcaaagccttggtgttgattgcctttgctcagtatcttcagcagtgtccatttgaagatcatgtaaaattagtgaatgaagtaactgaatttgcaaaaacatgtgttgctgatgagtcagctgaaaattgtgacaaatcacttcataccctttttggagacaaattatgcacagttgcaactcttcgtgaaacctatggtgaaatggctgactgctgtgcaaaacaagaacctgagagaaatgaatgcttcttgcaacacaaagatgacaacccaaacctcccccgattggtgagaccagaggttgatgtgatgtgcactgcttttcatgacaatgaagagacatttttgaaaaaatacttatatgaaattgccagaagacatccttacttttatgccccggaactccttttctttgctaaaaggtataaagctgcttttacagaatgttgccaagctgctgataaagctgcctgcctgttgccaaagctcgatgaacttcgggatgaagggaaggcttcgtctgccaaacagagactcaagtgtgccagtctccaaaaatttggagaaagagctttcaaagcatgggcagtagctcgcctgagccagagatttcccaaagctgagtttgcagaagtttccaagttagtgacagatcttaccaaagtccacacggaatgctgccatggagatctgcttgaatgtgctgatgacagggcggaccttgccaagtatatctgtgaaaatcaagattcgatctccagtaaactgaaggaatgctgtgaaaaacctctgttggaaaaatcccactgcattgccgaagtggaaaatgatgagatgcctgctgacttgccttcattagctgctgattttgttgaaagtaaggatgtttgcaaaaactatgctgaggcaaaggatgtcttcctgggcatgtttttgtatgaatatgcaagaaggcatcctgattactctgtcgtgctgctgctgagacttgccaagacatatgaaaccactctagagaagtgctgtgccgctgcagatcctcatgaatgctatgccaaagtgttcgatgaatttaaacctcttgtggaagagcctcagaatttaatcaaacaaaattgtgagctttttgagcagcttggagagtacaaattccagaatgcgctattagttcgttacaccaagaaagtaccccaagtgtcaactccaactcttgtagaggtctcaagaaacctaggaaaagtgggcagcaaatgttgtaaacatcctgaagcaaaaagaatgccctgtgcagaagactatctatccgtggtcctgaaccagttatgtgtgttgcatgagaaaacgccagtaagtgacagagtcaccaaatgctgcacagaatccttggtgaacaggcgaccatgcttttcagctctggaagtcgatgaaacatacgttcccaaagagtttaatgctgaaacattcaccttccatgcagatatatgcacactttctgagaaggagagacaaatcaagaaacaaactgcacttgttgagctcgtgaaacacaagcccaaggcaacaaaagagcaactgaaagctgttatggatgatttcgcagcttttgtagagaagtgctgcaaggctgacgataaggagacctgctttgccgaggagggtaaaaaacttgttgctgcaagtcaagctgccttaggctta

SEQ ID NO: 51 - protein, 4 aa, Artificial Sequence
  Short flexible linker
GSGS

SEQ ID NO: 52 - protein, 5 aa, Artificial Sequence
  Short flexible linker
GSGSA

SEQ ID NO: 53 - protein, 15 aa, Artificial Sequence
  Long flexible linker
GGGGSGGGGSGGGGS

SEQ ID NO: 54 - protein, 227 aa, Artificial Sequence
  Fusion protein
DKTHTCPPCPAPEAAGGPSVFLFPPKPKDTLMISRTPEVTCVVVDVSHEDPEVKFNWYVDGVEVHNAKTKPREEQYNSTYRVVSVLTVLHQDWLNGKEYKCKVSNKALGAPIEKTISKAKGQPREPQVYTLPPSRDELTKNQVSLTCLVKGFYPSDIAVEWESNGQPENNYKTTPPVLDSDGSFFLYSKLTVDKSRWQQGNVFSCSVMHEALHNHYTQKSLSLSPGK

SEQ ID NO: 55 - protein, 229 aa, Artificial Sequence
  Fusion protein
ESKYGPPCPPCPAPEFLGGPSVFLFPPKPKDTLMISRTPEVTCVVVDVSQEDPEVQFNWYVDGVEVHNAKTKPREEQFNSTYRVVSVLTVLHQDWLNGKEYKCKVSNKGLPSSIEKTISKAKGQPREPQVYTLPPSQEEMTKNQVSLTCLVKGFYPSDIAVEWESNGQPENNYKTTPPVLDSDGSFFLYSRLTVDKSRWQEGNVFSCSVMHEALHNHYTQKSLSLSLGK

SEQ ID NO: 56 - protein, 6 aa, Artificial Sequence
  Six His peptide
HHHHHH

SEQ ID NO: 57 - protein, 8 aa, Artificial Sequence
  Strp-Tactin binding peptide
WSHPQFEK

SEQ ID NO: 58 - protein, 585 aa, Homo sapiens [sequence omitted]

SEQ ID NO: 59 - protein, 669 aa, Artificial Sequence
  Fusion protein
SGDAHKSEVAHRFKDLGEENFKALVLIAFAQYLQQCPFEDHVKLVNEVTEFAKTCVADESAENCDKSLHTLFGDKLCTVATLRETYGEMADCCAKQEPERNECFLQHKDDNPNLPRLVRPEVDVMCTAFHDNEETFLKKYLYEIARRHPYFYAPELLFFAKRYKAAFTECCQAADKAACLLPKLDELRDEGKASSAKQRLKCASLQKFGERAFKAWAVARLSQRFPKAEFAEVSKLVTDLTKVHTECCHGDLLECADDRADLAKYICENQDSISSKLKECCEKPLLEKSHCIAEVENDEMPADLPSLAADFVESKDVCKNYAEAKDVFLGMFLYEYARRHPDYSVVLLLRLAKTYETTLEKCCAAADPHECYAKVFDEFKPLVEEPQNLIKQNCELFEQLGEYKFQNALLVRYTKKVPQVSTPTLVEVSRNLGKVGSKCCKHPEAKRMPCAEDYLSVVLNQLCVLHEKTPVSDRVTKCCTESLVNRRPCFSALEVDETYVPKEFNAETFTFHADICTLSEKERQIKKQTALVELVKHKPKATKEQLKAVMDDFAAFVEKCCKADDKETCFAEEGKKLVAASQAALGLGGGGSGGGGSGGGGSAYRPSETLCGGELVDTLQFVCGDRGFYFSRPASRVSARSRGIVEECCFRSCDLALLETYCATPAKSE

SEQ ID NO: 60 - protein, 675 aa, Artificial Sequence
  Fusion protein
RGVFRRSGDAHKSEVAHRFKDLGEENFKALVLIAFAQYLQQCPFEDHVKLVNEVTEFAKTCVADESAENCDKSLHTLFGDKLCTVATLRETYGEMADCCAKQEPERNECFLQHKDDNPNLPRLVRPEVDVMCTAFHDNEETFLKKYLYEIARRHPYFYAPELLFFAKRYKAAFTECCQAADKAACLLPKLDELRDEGKASSAKQRLKCASLQKFGERAFKAWAVARLSQRFPKAEFAEVSKLVTDLTKVHTECCHGDLLECADDRADLAKYICENQDSISSKLKECCEKPLLEKSHCIAEVENDEMPADLPSLAADFVESKDVCKNYAEAKDVFLGMFLYEYARRHPDYSVVLLLRLAKTYETTLEKCCAAADPHECYAKVFDEFKPLVEEPQNLIKQNCELFEQLGEYKFQNALLVRYTKKVPQVSTPTLVEVSRNLGKVGSKCCKHPEAKRMPCAEDYLSVVLNQLCVLHEKTPVSDRVTKCCTESLVNRRPCFSALEVDETYVPKEFNAETFTFHADICTLSEKERQIKKQTALVELVKHKPKATKEQLKAVMDDFAAFVEKCCKADDKETCFAEEGKKLVAASQAALGLGGGGSGGGGSGGGGSAYRPSETLCGGELVDTLQFVCGDRGFYFSRPASRVSARSRGIVEECCFRSCDLALLETYCATPAKSE